European Patent Specification EP 3 824 285 B1, published December 11, 2024. Title: MOLECULAR HOPPER. Applicant: Oxford University Innovation Limited. The sequence listing filed with the application follows.

SEQUENCE LISTING (15 sequences)

SEQ ID NO: 1 - protein, 293 aa, Staphylococcus aureus
ADSDINIKTGTTDIGSNTTVKTGDLVTYDKENGMHKKVFYSFIDDKNHNKKLLVIRTKGTIAGQYRVYSEEGANKSGLAWPSAFKVQLQLPDNEVAQISDYYPRNSIDTKEYMSTLTYGFNGNVTGDDTGKIGGLIGANVSIGHTLKYVQPDFKTILESPTDKKVGWKVIFNNMVNQNWGPYDRDSWNPVYGNQLFMKTRNGSMKAADNFLDPNKASSLLSSGFSPDFATVITMDRKASKQQTNIDVIYERVRDDYQLHWTSTNWKGTNTKDKWTDRSSERYKIDWEKEEMTN

SEQ ID NO: 2 - protein, 307 aa, Artificial Sequence
  alpha hemolysin mutant (WT-D8H6)
ADSDINIKTGTTDIGSNTTVKTGDLVTYDKENGMHKKVFYSFIDDKNHNKKLLVIRTKGTIAGQYRVYSEEGANKSGLAWPSAFKVQLQLPDNEVAQISDYYPRNSIDTKEYMSTLTYGFNGNVTGDDTGKIGGLIGANVSIGHTLKYVQPDFKTILESPTDKKVGWKVIFNNMVNQNWGPYDRDSWNPVYGNQLFMKTRNGSMKAADNFLDPNKASSLLSSGFSPDFATVITMDRKASKQQTNIDVIYERVRDDYQLHWTSTNWKGTNTKDKWTDRSSERYKIDWEKEEMTNDDDDDDDDHHHHHH

SEQ ID NO: 3 - protein, 307 aa, Artificial Sequence
  alpha hemolysin mutant (115C117C-D8H6)
ADSDINIKTGTTDIGSNTTVKTGDLVTYDKENGMHKKVFYSFIDDKNHNKKLLVIRTKGTIAGQYRVYSEEGANKSGLAWPSAFKVQLQLPDNEVAQISDYYPRNSIDTKEYMSCLCYGFNGNVTGDDTGKIGGLIGANVSIGHTLKYVQPDFKTILESPTDKKVGWKVIFNNMVNQNWGPYDRDSWNPVYGNQLFMKTRNGSMKAADNFLDPNKASSLLSSGFSPDFATVITMDRKASKQQTNIDVIYERVRDDYQLHWTSTNWKGTNTKDKWTDRSSERYKIDWEKEEMTNDDDDDDDDHHHHHH

SEQ ID NO: 4 - protein, 307 aa, Artificial Sequence
  alpha hemolysin mutant (115C117C119C-D8H6)
ADSDINIKTGTTDIGSNTTVKTGDLVTYDKENGMHKKVFYSFIDDKNHNKKLLVIRTKGTIAGQYRVYSEEGANKSGLAWPSAFKVQLQLPDNEVAQISDYYPRNSIDTKEYMSCLCYCFNGNVTGDDTGKIGGLIGANVSIGHTLKYVQPDFKTILESPTDKKVGWKVIFNNMVNQNWGPYDRDSWNPVYGNQLFMKTRNGSMKAADNFLDPNKASSLLSSGFSPDFATVITMDRKASKQQTNIDVIYERVRDDYQLHWTSTNWKGTNTKDKWTDRSSERYKIDWEKEEMTNDDDDDDDDHHHHHH

SEQ ID NO: 5 - protein, 307 aa, Artificial Sequence
  alpha hemolysin mutant (113C115C117C119C121C-D8H6)
ADSDINIKTGTTDIGSNTTVKTGDLVTYDKENGMHKKVFYSFIDDKNHNKKLLVIRTKGTIAGQYRVYSEEGANKSGLAWPSAFKVQLQLPDNEVAQISDYYPRNSIDTKEYCSCLCYCFCGNVTGDDTGKIGGLIGANVSIGHTLKYVQPDFKTILESPTDKKVGWKVIFNNMVNQNWGPYDRDSWNPVYGNQLFMKTRNGSMKAADNFLDPNKASSLLSSGFSPDFATVITMDRKASKQQTNIDVIYERVRDDYQLHWTSTNWKGTNTKDKWTDRSSERYKIDWEKEEMTNDDDDDDDDHHHHHH

SEQ ID NO: 6 - protein, 307 aa, Artificial Sequence
  alpha hemolysin mutant (113C115C117C119C121C123C-D8H6)
ADSDINIKTGTTDIGSNTTVKTGDLVTYDKENGMHKKVFYSFIDDKNHNKKLLVIRTKGTIAGQYRVYSEEGANKSGLAWPSAFKVQLQLPDNEVAQISDYYPRNSIDTKEYCSCLCYCFCGCVTGDDTGKIGGLIGANVSIGHTLKYVQPDFKTILESPTDKKVGWKVIFNNMVNQNWGPYDRDSWNPVYGNQLFMKTRNGSMKAADNFLDPNKASSLLSSGFSPDFATVITMDRKASKQQTNIDVIYERVRDDYQLHWTSTNWKGTNTKDKWTDRSSERYKIDWEKEEMTNDDDDDDDDHHHHHH

SEQ ID NO: 7 - protein, 307 aa, Artificial Sequence
  alpha hemolysin mutant (115C117C119C139C-D8H6)
ADSDINIKTGTTDIGSNTTVKTGDLVTYDKENGMHKKVFYSFIDDKNHNKKLLVIRTKGTIAGQYRVYSEEGANKSGLAWPSAFKVQLQLPDNEVAQISDYYPRNSIDTKEYMSCLCYCFNGNVTGDDTGKIGGLIGACVSIGHTLKYVQPDFKTILESPTDKKVGWKVIFNNMVNQNWGPYDRDSWNPVYGNQLFMKTRNGSMKAADNFLDPNKASSLLSSGFSPDFATVITMDRKASKQQTNIDVIYERVRDDYQLHWTSTNWKGTNTKDKWTDRSSERYKIDWEKEEMTNDDDDDDDDHHHHHH

SEQ ID NO: 8 - DNA, 36 bp, Artificial Sequence
  forward mutagenic primer
ctgcttctgcggttgtgttactggtgatgatacagg

SEQ ID NO: 9 - DNA, 23 bp, Artificial Sequence
  reverse non-mutagenic primer (SC47)
cagaagtggtcctgcaactttat

SEQ ID NO: 10 - DNA, 36 bp, Artificial Sequence
  reverse mutagenic primer
cctgtatcatcaccagtaacacaaccgcagaagcag

SEQ ID NO: 11 - DNA, 23 bp, Artificial Sequence
  forward non-mutagenic primer (SC46)
ataaagttgcaggaccacttctg

SEQ ID NO: 12 - DNA, 39 bp, Artificial Sequence
  forward mutagenic primer
caaaagagtatatgagttgcttatgctattgcttcaacg

SEQ ID NO: 13 - DNA, 39 bp, Artificial Sequence
  reverse mutagenic primer
cgttgaagcaatagcataagcaactcatatactcttttg

SEQ ID NO: 14 - DNA, 37 bp, Artificial Sequence
  forward mutagenic primer
ccttattggtgcatgtgtttcgattggtcatacactg

SEQ ID NO: 15 - DNA, 37 bp, Artificial Sequence
  reverse mutagenic primer
cagtgtatgaccaatcgaaacacatgcaccaataagg